European Patent Specification EP 3 732 293 B1, published July 3, 2024. Title: Optimiertes Wirts-/Vektorsystem zur Erzeugung protektiver mono- und multivalenter subunit-Vakzine auf Basis der Hefe Kluyveromyces lactis. Applicant: Martin-Luther-Universität Halle-Wittenberg. The sequence listing filed with the application follows.

SEQUENCE LISTING (25 sequences)

SEQ ID NO: 1 - DNA, 5042 bp, Kluyveromyces lactis
atgaatatcaatatcaagaaagattctggagggaatgggtccgatttacctcgatggaacgattctccggtgggaagtttagggtcgtttaatgggagaagaagatcgatgtccttctctgaatcagtaaacttcgcaagaaatactcagaacccattggatatgtcagctcaggaaatgagaggattgaatgggttcagaagatctttcatcgctcataagtcgttgaaacttcatgggaagacaccgaactttatcactaggaatttcaacgagttcttgacgttatacggccatttcgctggtgaagatttgtccgaggatgaggaaacagaaactgaggtggagactgatgaagatgaggacgaagaagctgcgcttcttcgtcatggtattaggggcctgcgccacctcgacaatttcaaacgtatcagagtgctttgccaattgttcggcagcagtcttcatacctcttacgatggcagggtatggcgttacaaggttatcagtatataggacaccgaccttgatcttctgaggcagttcagcttctctccaaggaatagggatactagtagtatcagattcccaaggcttaccgtcattaatgtaatgtttcataaagtaatccagctcttcaatagatcctctacgccggacgcatcgtggccggcatcaccggcgccacaggtgcggttgctggcgcctatatcgccgacatcaccgatggggaagatcgggctcgccacttcgggctcatgagcgcttgtttcggcgtgggtatggtggcaggccccgtggccgggggactgttgggcgccatctccttgcatgcaccattccttgcggcggcggtgctcaacggcctcaacctactactgggctgcttcctaatgcaggagtcgcataagggagagcgtcgatcgacctttgacattcgctgttcaaagttaccacagcagcaattgatccaagctaactcacggcacgggcgtagcaagtgaaccgtcgatattgagcagtgtatgaatatgcattcgtaccagtattttgtgtgatcacgcaggactttacggtttcacggaccggaacagaccgtattcctgtccttaagtgtaatgtatgggtgtgatctctgtcctccgcctttcccatacaaaagttgctttgaaaaagaagtaactgcaaaatcatagataatgacactttgaataactagaaataacaacttcggacccttgctcaattcaagtaagacaatatatagcgtacctgccgttcttccaagtgagggtttgttctgttggttcagaaatcccaggatattcagagttttttaaagcttttcttagagtcaaggcacttttttacaccaattgtactagtacccaactaaacattaaaagatcagcaaccatccaaatggtttacgatttgaccatttgaacatcacagatctgaactttactccgactgattgtttttactatacgaaatgggtagtagggcctccaattcgccttctttttcaagtaaggcggaaacgttactgccatcggagtataaaaagaatgcggttaagaaggaaacaatacgcaatggcaagaaaaggaaattgcctgatacagaatcctcagatcctgagtttgcaagtcggcgtttgatagctaatgaaactggcactgatgcggtgagtaatggtaacaaaaatgatagcaatgccaacaacaacaacaacaacaacaacaagaaatcaagtgaagtaatgcaccaggcgtgcgatgcttgcaggaagaagaagtggaaatgttccaagacagtaccgacttgcacgaactgtctgaaatacaatttagactgtgtctactctccgcaagttgttaggactccgttgacaagagcacatttaacagagatggaaaatagggttgcagagttggaacagtttttgaaagaacttttcccagtttgggatatcgataggttacttcagcaaaaagatacatacaggattagggaattgcttactatgggttctacaaatactgttccgggacttgcatcgaataatatcgattcatcgttagaacagcccgttgcctttggtactgcgcagccggcacaatctttgtcaactgatccagcagtacaatctcaagcctatccaatgcaaccggtaccgatgacagagcttcaatctatcaccaatcttcgacacacgccatcacttctggatgaacagcaaatgaacacgatttccacggcaacgctgcggaacatgtactcttcaggtaacaataataacaacttgggtaacatctctggtctatcacctgttacagaggcattcttccgttggcaggaaggtgaaacgtcaatcgataatagttattttggaaaaggttcaattttgttttggttgaaccaattactatcatcagaaaagatcgctggcgttacatcaaaagtaggcaatgacattaacactaataataataatataaaccatcagaagctacctctaatactaaacaataatattactcataatgtgtcggacataaccacaacaagtacatcttcaaacaaaagggcaatgtctcctctttctgccaatgactctgtatatctcgctaaaagagagacaatatccgcgtatatcgatgcgtacttcaagcactatcatgcgctatatccgttggtcagtaaggaaatgtttttcgctcagtataatgatcaaattaaaccagagaacgttgagatatggcacatcttactaaacgcggtattagctttgggttcatggtgctctaattcatgttcaagtcaccatactctctattaccaaaacgcattatcatatttgtccaccgctgtattggaaacagggtccacagatttaaccatagcactcatacttttaacgcattatgttcaaaagatgcataagccaaacactgcatggagtctcataggactttgtagccatatggctacatcgttgggattacaccgggatctaccaaactcaacgatacatgatcagcaactccgtagagtattgtggtggactatttattgcacgggatgcgatctctcattagagactggaaggccctcattattgcccaatcttcaggctattgatataccattaccagcttcatctgccactatcaaagaaccaagcatatattcctccatcatacaagaatcccaatggtctcaaatattgcaacagaaattgtcaaataactcatatcagcaaagtgcaggtgaatgtctctcatggttcgatagtgttcaagcatttttagaccactggcctactcctagtaccgaagctgaactcaaagccttaaatgaaactcaactagattggctaccattagtgaagttccggccatactggatgttccattgttccctaatatcacttttctcagttttttttgaagaagatgccccaaccgacaacaacgtcatacggtgcaaggagttatgccttcaactttcaagcagaaatatatttagcgtggccacttttgtacggagctatgcattcaactcactttcctgttggtacgcgacacattatcttgttagaagcgcattagtgcctctacatttcgcatctcggatatctccacagcacgccttgtgggagacagttaaagcgcaattattatcagcccatgaagcgatgggtatattgtcacaagaatcttccttggccgctaaatttgatgggatattaaccaagaattattctgaaatactacaaagagaaggcatcaacaaaagccaactgatgccaccaccaactccattgctacaatcaaccagtttctcggacctactttcactgtggtcagcaaacgcagaagacgctccgagagtcagtaattcccagatgcctcaatcgatcactatcacggactctttgctacagtcatcaacaactcaaatgagacctccaaccacatctggatggcctgataccaacaacttcctgaatccatcgacccaacagctattcaacaccacaacaatggacgatgtgtacaactatatatttgataacgacgagtaagaaatctctcttttccgtagtcaattgggacagcatcaattcatgtatttactttttgttcagtagctatcaaatagctatccaacgagaccactggtacgaacagtgtccatcatgcacattgtaggtaacccagggagcggatcggtatggcgaagagacttcatcgatggccatcgatgatgacgaaggtagttcggaaaataacgatatccagcaacaacagcagctgaagcagcagcagcagcacttgcataagaagaaaagaaatacgtccaccacgaaggcggtacttctccttctaaagtcgttcgtaggtaccggggttctttttctacctagagctttccataacggtgggtggttgttcagtacgctgtgtcttttgttctgcgccacggtgtctttctactgcttcatcctgttgatagacacgaagactgctgttggagtggatggatacggtgaattgggttcacgtttattcggacccaaattgaagttcactgtcctttcatcgattgtactctcgcaaatcggatttgctgctgcttatactgtgttcactgcaacaaacttgcaggcattcttcaaacatgtcttttctctcgaatactcgttaatcttctggattatgatccaactagcattctatttgccgctatcattgactagaaacattgcaagactcagtgccaccgctttggtagcagatcttttcattctcttgggtctagtatacgtctattattattccagtttctatatttggaaccatggcatcgcttcggattccatggtgtctttcaacaaatcggactggacgttatttattggaactgcgatattcacatatgagggtatcggtctcttgatcccaatccatgaatctatggaaaaacctgcacatttcaaaccggcattgatgtacgtcatcctcgttgtaaca

SEQ ID NO: 2 - DNA, 2349 bp, Artifizielle Sequenz
  Synthetische Polynukleinsäure
cgtaattctgtctttaatcattaacactgactgaaggatataattataagacaacacacagagacttttgtttgctgtttagcttacactttccagctatattgaatagcatatatatgttccagaagctacaaccaccttgaactacagcccaactcaacattgaaagttactgcctttatataccttgatacaccatttagacctccaattaaccgattgtccttgtcataatgagctagagtagcaaggtatcaacaacagtatggacatcttattgtcaactttctagtacggagggaagaatcccgaatatgttaaatctgacgcgcgggtattgctaagtcacgttgcaggcccacgcagacccgagtttctttcttacaaaagcgtgtacacacgtaaacgcgctcggtgcaccgaacggccagggtcggggttcattcggtatagagccacgcaggtaacttgccaattccaaaaaaaattaaatgacgatactagtaaccaaaggaaaggaacagatagataaaattccgagactgtcaaattaggtttttttctttttttttggcgggagtcagtgggccgaaatatgttcttggcctagaacttaatctggtttgatcatgccaatacttgcctgagtgcccgactttttgcccaccctcttgccttctgtctatccttcaaaacccacctgttttccagccgtatcttcgctcgcatctacacatactgtgccatatcttgtgtgtagccggacgtgactatgaccaaaaacaaacaaggagaactgttcgccgatttgtaacactcctgcatccatccaagtgggtatgcgctatgcaatgttaagctaggtcaggtcagaccaggtccaaggacagcaacttgactgtatgcaacctttaccatctttgcacagaacatacttgtagctagctagttacacttatggaccgaaaaggcaccccaccatgtctgtccggctttagagtacggccgcagaccgctgatttgccttgccaagcagtagtcacaatgcatcgcatgagcacacgggcacgggcacgggcacaggaaccattggcaaaaataccagatacactataccgacgtatatcaagcccaagtttaaaattcctaaatttccgcggggatcgactcataaaatagtaaccttctaatgcgtatctattgactaccaaccattagtgtggttgcagaaggcggaattcgtcgacgaacttgtttaattattatggggcaggcgagagggggaggaatgtatgtgtgtgaggcgggcgagacggagccatccaggccaggtagaaatagagaaagccgaatgttagacaatatggcagcgtagtagagtaggtaggtaggcaagtactgctagcaaagaggagaagggtaagctcactcttcgcattccacaccgttagtgtgtcagtttgaacaaaaaaacaatcatcataccaattgatggactgtggactggcttttggaacggcttttcggactgcgattattcgtgaggaatcaaggtaggaatttggtcatatttacggacaacagtgggtgattcccatatggagtaggaaaacgagatcatggtatcctcagatatgttgcggaattctgttcaccgcaaagttcagggtgctctggtgggtttcggttggtctttgctttgcttctcccttgtcttgcatgttaataatagcctagcctgtgagccgaaacttagggtaggcttagtgttggaacgtacatatgtatcacgttgacttggtttaaccaggcgacctggtagccagccatacccacacacgttttttgtatcttcagtatagttgtgaaaagtgtagcggaaatttgtggtccgagcaacagcgtctttttctagtagtgcggtcggttacttggttgacattggtatttggactttgttgctacaccattcactacttgaagtcgagtgtgaagggtatgatttctagtggtgaacacctttagttacgtaatgttttcattgctgttttacttgagatttcgattgagaaaaaggtatttaatagctcgaatcaatgtgagaacagagagaggatgttcttccctaactcgaaaggtatatgaggcttgtgtttcttaggagaattattattcttttgttatgttgcgcttgtagttggaaaaggtgaagagacaaaagctggaattgtgagcggataacaagctcaacacttgaaatttaggaaagagcagaatttggcaaaaaaaataaaaaaaaaataaacacacatactcatcgagaagctgtaccgtcgacggcgcgccatg

SEQ ID NO: 3 - DNA, 7964 bp, Artifizielle Sequenz
  Synthetische Polynukleinsäure
  Variation (6628)..(6629): nn ist aa, ag oder ga
aggtggcacttttcggggaaatgtgcgcggaacccctatttgtttatttttctaaatacattcaaatatgtatccgctcatgagacaataaccctgataaatgcttcaataatattgaaaaaggaagagtatgagtattcaacatttccgtgtcgcccttattcccttttttgcggcattttgccttcctgtttttgctcacccagaaacgctggtgaaagtaaaagatgctgaagatcagttgggtgcacgagtgggttacatcgaactggatctcaacagcggtaagatccttgagagttttcgccccgaagaacgttttccaatgatgagcacttttaaagttctgctatgtggcgcggtattatcccgtattgacgccgggcaagagcaactcggtcgccgcatacactattctcagaatgacttggttgagtactcaccagtcacagaaaagcatcttacggatggcatgacagtaagagaattatgcagtgctgccataaccatgagtgataacactgcggccaacttacttctgacaacgatcggaggaccgaaggagctaaccgcttttttgcacaacatgggggatcatgtaactcgccttgatcgttgggaaccggagctgaatgaagccataccaaacgacgagcgtgacaccacgatgcctgtagcaatggcaacaacgttgcgcaaactattaactggcgaactacttactctagcttcccggcaacaattaatagactggatggaggcggataaagttgcaggaccacttctgcgctcggcccttccggctggctggtttattgctgataaatctggagccggtgagcgtgggtctcgcggtatcattgcagcactggggccagatggtaagccctcccgtatcgtagttatctacacgacggggagtcaggcaactatggatgaacgaaatagacagatcgctgagataggtgcctcactgattaagcattggtaactgtcagaccaagtttactcatatatactttagattgatttaaaacttcatttttaatttaaaaggatctaggtgaagatcctttttgataatctcatgaccaaaatcccttaacgtgagttttcgttccactgagcgtcagaccccgtagaaaagatcaaaggatcttcttgagatcctttttttctgcgcgtaatctgctgcttgcaaacaaaaaaaccaccgctaccagcggtggtttgtttgccggatcaagagctaccaactctttttccgaaggtaactggcttcagcagagcgcagataccaaatactgttcttctagtgtagccgtagttaggccaccacttcaagaactctgtagcaccgcctacatacctcgctctgctaatcctgttaccagtggctgctgccagtggcgataagtcgtgtcttaccgggttggactcaagacgatagttaccggataaggcgcagcggtcgggctgaacggggggttcgtgcacacagcccagcttggagcgaacgacctacaccgaactgagatacctacagcgtgagctatgagaaagcgccacgcttcccgaagggagaaaggcggacaggtatccggtaagcggcagggtcggaacaggagagcgcacgagggagcttccagggggaaacgcctggtatctttatagtcctgtcgggtttcgccacctctgacttgagcgtcgatttttgtgatgctcgtcaggggggcggagcctatggaaaaacgccagcaacgcggcctttttacggttcctggccttttgctggccttttgctcacatgttctttcctgcgttatcccctgattctgtggataaccgtattaccgcctttgagtgagctgataccgctcgccgcagccgaacgaccgagcgcagcgagtcagtgagcgaggaagcggaagagcgcccaatacgcaaaccgcctctccccgcgcgttggccgattcattaatgcagctggcacgacaggtttcccgactggaaagcgggcagtgagcgcaacgcaattaatgtgagttagctcactcattaggcaccccaggctttacactttatgctcccggctcgtatgttgtgtggaattgtgagcggataacaatttcacacaggaaacagctatgaccatgattacgccaagcgcgcaattaaccctcactaaagggaacaaaagctgggtaccgggcccggtgacctcattgcagtcgtttatactcctcaggagaacgcagttgcgacctcatataatcaagcaaaagaagaccggcagtagttccaggaataattgccaaagtattcctagtaaaacctttatataaccaagcaatggtttctctcttacttctcttcatgaaaaagaacacatgctcgaatgtatccaagtatgagttgtaatagatgtgaaacctactactgcctttgggtatccttattttcgtatttggaatatttcctatagttgtactagacgttgatggtagatttttgagataaatatcgtacgcttcaagtctagagacgtggattttctgtagctttaggaacgggaattgcaccgattgaagaacaaaagctgctgtaacacctccaataaaaatgaaaactcttgaataccacatttcctctttaggagaaattaaccttggtttcttcgtttcaatcttattaccatcttcatcgaaaaatatatccgagagtcttgtgttctgcaccgtatattttagttccctataattcttgataaaatctaacatcaattggcgaattggtcctctgatcatttcaaaagtagtgaaatacaatgcaaagccaaaggattctcttatgaatgataatccaaacccaccaaagcagccaatcaaaccaatctctctgatcttatcacgactataaagccatagattatcatatttttttgcgctggataaaagttcatcaatgtttgctcttgtataaatggcatctattggagctgagacaatggcttgtgcagcacctgcaaggaatcctgctcttaaaaaatcaaacatattatgttgaaaagcttgatctgtagccctcaacggaaaattattcaaagtggctaaataagtagtgtatagcacaactcccgccagcgaattggctactaatggcggtaaaattctgtcaggtatgactttccaaccatatctgttcaatgctttagtgacgattccgattgaagagttctccaaataataagtatactttggattccaaaaccgatacctcgaacttcgtacttttgtctcggactgtgtattatcgctacctgtaagaagtactcgaatgtaatgagtatagtcaaatctagctggtctgaacaattttaacggagtcctcatgtaaaaagatgttagttgatacaccatagatcttccaccagcagtagcagcacccacaagagaagaggtttggtttgataatgaattgacatttgctttatctgaaacatcttccaatctcttgttggcatcagaagacatcactgtctcttccccttaatgatcacttgaacaaaactccgatagggtatagtcaatatgtgaaactggacactatatcaaagcaaaaagtagtgttggatgctaaatgggatcgttttatttaggttctatcgaggagaaaaagcgacaagaagagatagaccatggataaatgattatgttctaaacactcctcagaagctcatcgaactgtcatcctgcgtgaagattaaaatccaacttagaaatttcgagcttcgaaccgcggcccgggctcgagcgtaattctgtctttaatcattaacactgactgaaggatataattataagacaacacacagagacttttgtttgctgtttagcttacactttccagctatattgaatagcatatatatgttccagaagctacaaccaccttgaactacagcccaactcaacattgaaagttactgcctttatataccttgatacaccatttagacctccaattaaccgattgtccttgtcataatgagctagagtagcaaggtatcaacaacagtatggacatcttattgtcaactttctagtacggagggaagaatcccgaatatgttaaatctgacgcgcgggtattgctaagtcacgttgcaggcccacgcagacccgagtttctttcttacaaaagcgtgtacacacgtaaacgcgctcggtgcaccgaacggccagggtcggggttcattcggtatagagccacgcaggtaacttgccaattccaaaaaaaattaaatgacgatactagtaaccaaaggaaaggaacagatagataaaattccgagactgtcaaattaggtttttttctttttttttggcgggagtcagtgggccgaaatatgttcttggcctagaacttaatctggtttgatcatgccaatacttgcctgagtgcccgactttttgcccaccctcttgccttctgtctatccttcaaaacccacctgttttccagccgtatcttcgctcgcatctacacatactgtgccatatcttgtgtgtagccggacgtgactatgaccaaaaacaaacaaggagaactgttcgccgatttgtaacactcctgcatccatccaagtgggtatgcgctatgcaatgttaagctaggtcaggtcagaccaggtccaaggacagcaacttgactgtatgcaacctttaccatctttgcacagaacatacttgtagctagctagttacacttatggaccgaaaaggcaccccaccatgtctgtccggctttagagtacggccgcagaccgctgatttgccttgccaagcagtagtcacaatgcatcgcatgagcacacgggcacgggcacgggcacaggaaccattggcaaaaataccagatacactataccgacgtatatcaagcccaagtttaaaattcctaaatttccgcggggatcgactcataaaatagtaaccttctaatgcgtatctattgactaccaaccattagtgtggttgcagaaggcggaattctcccttcttcgaattcagcttgctttttcattttttattttccatttttcagtttttgtttgtgtcgaatttagccagttgcttctccaagatgaaaaaaacccctgcgcagtttctgtgctgcaagatcctaatcgacttttccaccccccacaaaagtaaatgttcttttgttacattcgcgtgggtagctagctccccgaatcttcaaaggacttagggactgcactacatcagagtgtgttcacctggtttgctgcctggtttgaaagaaaagagcagggaactcgcgggttcccggcgaataatcatgcgatagtcctttggccttccaagtcacatgtagagtagacaacagacagggagggcaggaaggatctttcactgagatcctgtatcttgttgggtaagtcggatgaaaggggaatcgtatgagattggagaggatgcggaagaggtaacgccttttgttaacttgtttaattattatggggcaggcgagagggggaggaatgtatgtgtgtgaggcgggcgagacggagccatccaggccaggtagaaatagagaaagccgaatgttagacaatatggcagcgtagtagagtaggtaggtaggcaagtactgctagcaaagaggagaagggtaagctcactcttcgcattccacaccgttagtgtgtcagtttgaacaaaaaaacaatcatcataccaattgatggactgtggactggcttttggaacggcttttcggactgcgattattcgtgaggaatcaaggtaggaatttggtcatatttacggacaacagtgggtgattcccatatggagtaggaaaacgagatcatggtatcctcagatatgttgcggaattctgttcaccgcaaagttcagggtgctctggtgggtttcggttggtctttgctttgcttctcccttgtcttgcatgttaataatagcctagcctgtgagccgaaacttagggtaggcttagtgttggaacgtacgtatgtatcacgttgacttggtttaaccaggcgacctggtagccagccatacccacacacgttttttgtatcttcagtatagttgtgaaaagtgtagcggaaatttgtggtccgagcaacagcgtctttttctagtagtgcggtcggttacttggttgacattggtatttggactttgttgctacaccattcactacttgaagtcgagtgtgaagggtatgatttctagtggtgaacacctttagttacgtaatgttttcattgctgttttacttgagatttcgattgagaaaaaggtatttaatagctcgaatcaatgtgagaacagagagaggatgttcttccctaactcgaaaggtatatgaggcttgtgtttcttaggagaattattattcttttgttatgttgcgcttgtagttggaaaaggtgaagagacaaaagctggaattgtgagcggataacaagctcaacacttgaaatttaggaaagagcagaatttggcaaaaaaaataaaaaaaaataaacacacatactcatcgagaagctgtaccgtcgacggcgcgccatgtnngcggccgcctcgactcagtactgacaataaaaagattcttgttttcaagaacttgtcatttgtatagtttttttatattgtagttgttctattttaatcaaatgttagcgtgatttatattttttttcgcctcgacatcatctgcccagatgcgaagttaagtgcgcagaaagtaatatcatgcgtcaatcgtatgtgaatgctggtcgctatactgctgtcgattcgatactaacgccgccatccagtgtcgaaaacgagctctcgacacgcgtcacaagcttcggagacaatcatatgggagaagcaattggaagatagaaaaaaggtactcggtacataaatatatgtgattctgggtagaagatcggtctgcattggatggtggtaacgcatttttttacacacattacttgcctcgagcatcaaatggtggttattcgtggatctatatcacgtgatttgcttaagaattgtcgttcatggtgacacttttagctttgacatgattaagctcatctcaattgatgttatctaaagtcatttcaactatctaagatgtggttgtgattgggccattttgtgaaagccagtacgccagcgtcaatacactcccgtcaattagttgcaccatgtccacaaaatcatataccagtagagctgagactcatgcaagtccggttgcatcgaaacttttacgtttaatggatgaaaagaagaccaatttgtgtgcttctcttgacgttcgttcgactgatgagctattgaaacttgttgaaacgttgggtccatacatttgccttttgaaaacacacgttgatatcttggatgatttcagttatgagggtactgtcgttccattgaaagcattggcagagaaatacaagttcttgatatttgaggacagaaaattcgccgatatcggtaacacagtcaaattacaatatacatcgggcgtttaccgtatcgcagaatggtctgatatcaccaacgcccacggggttactggtgctggtattgttgctggcttgaaacaaggtgcgcaagaggtcaccaaagaaccaaggggattattgatgcttgctgaattgtcttccaagggttctctagcacacggtgaatatactaagggtaccgagctccaattcgccctatagtgagtcgtattacgcgcgctcactggccgtcgttttacaacgtcgtgactgggaaaaccctggcgttacccaacttaatcgccttgcagcacatccccctttcgccagctggcgtaatagcgaagaggcccgcaccgatcgcccttcccaacagttgcgcagcctgaatggcgaatgg

SEQ ID NO: 4 - DNA, 9728 bp, Artifizielle Sequenz
  Synthetische Polynukleinsäure
  Variation (4962)..(4963): nn is aa, ag oder ga
tcagctctgggagaaacttggtgtttccggtgcaactgtccctgatgaaccaaagccgatcaccaatgaagatatcaaaattgcttccaatttcctcagaggtacaattgtggaagggctacaagatgaatcaactggtgcaatttctgcgtgggatcagcaattaaccaagttccatggtatctatatgcaagatgatcgtgatataagagacactaggaagagtcaaggtcttgaaccttattacattttcatgtcaagagttagattaccaggtggaaaggccaatccagatcaatggttgattcttgatcacttagcagacaaaactggtaacggtacagttaaaattaccaccagagcaactttccaattgcatggtgttgttaagcacaatttaaagcacactatcagagctatgaattccaccttgatggacactttagcggcgtgtggtgatgttaacagaaatgtcatgctttctgctttgcctgctaatgccacggttcacaaacaaattgcagacgttggtacatatctttctgaacgtttcttgcctcaaacaacggcgtatcacgaaatttggttagagggtccagacaaggatgatgaagatccttcttggccagagacctacgagaaaagacaagaaggtcctataaagaagaagaaaactcttgttgccggtaatgcattagttgatgcggaaccagtctatggtccaacatacttaccaagaaagttcaagatcaatattactgttccacctttcaatgatgtcgatgtgtggtccagtgacgttggtttgattgctataattgatgaaccaactcaaactctaacaggtttcaatctctatgttggtggtggtatggggagtacccacaacaacaaaaagacatacccaagaacaggttcgttgttcgggtatgtctccgtagcagatgtgggagatgccattgaaaaggtgatgattgttcaaagagatcatggtgatcgtaccaaccgtaagcacgctcgtttaaagtacactgttgatgatttgaccattgaaggttacaagcagaaggtcgaagaactatggggcaagaagtttgaacctgctgctgcgtatgagatcaaatcaaacattgattacttcggttgggtaaaggatgaaactggactaaatcatttcactgccttcattgaaaatggtagagtggaagatacagtagagctgcctcagaaaacaggtttcaggaaaattgcacagttgatgaagaaagataacttcggtcacttcagattaaccggtaaccaacacgttcttatctcagacgttgatgacgagcatttagacgaagttaaagctatcatgaacaagtacaagctagacaacacgaacttcagtggattgaggttatcgtctgctgcatgtgttgctttgccaacctgtggtttggctatggccgaatctgaacgttatttgcctgttttaatcacaaagctggagaatgcattagaagagtatgggttacgccacgattctattgtcatgagaatgactggttgtccaaatggttgtgctcgtccatggttagctgaggttgctttagtgggtaaagccccaggaacttataatctattactcggaggtggttattacggtcaaagattgaacaaactatacagagcatccatcaaagaagatgaaattttagccacattgaaacctctatttaagaggtggtccttggaaagactcgaaggtgaacacttcggggatttcgtcattagagtaggtgttatcaaaccaaccttggaaggtaaatacttccatgatgatcttccagaagaagctctatgagggagccaactcctttcatatgggagggccgcatcatgtaattagttatgtcacgcttacattcacgccctccccccacatccgctctaaccgaaaaggaaggagttagacaacctgaagtctaggtccctatttatttttttatagttatgttagtattaagaacgttatttatatttcaaatttttcttttttttctgtacagacgcgtgtacgcatgtaacattatactgaaaaccttgcttgagaaggttttgggacgctcgaaggctttaatttgcggcccccgggctcgagcgtaattctgtctttaatcattaacactgactgaaggatataattataagacaacacacagagacttttgtttgctgtttagcttacactttccagctatattgaatagcatatatatgttccagaagctacaaccaccttgaactacagcccaactcaacattgaaagttactgcctttatataccttgatacaccatttagacctccaattaaccgattgtccttgtcataatgagctagagtagcaaggtatcaacaacagtatggacatcttattgtcaactttctagtacggagggaagaatcccgaatatgttaaatctgacgcgcgggtattgctaagtcacgttgcaggcccacgcagacccgagtttctttcttacaaaagcgtgtacacacgtaaacgcgctcggtgcaccgaacggccagggtcggggttcattcggtatagagccacgcaggtaacttgccaattccaaaaaaaattaaatgacgatactagtaaccaaaggaaaggaacagatagataaaattccgagactgtcaaattaggtttttttctttttttttggcgggagtcagtgggccgaaatatgttcttggcctagaacttaatctggtttgatcatgccaatacttgcctgagtgcccgactttttgcccaccctcttgccttctgtctatccttcaaaacccacctgttttccagccgtatcttcgctcgcatctacacatactgtgccatatcttgtgtgtagccggacgtgactatgaccaaaaacaaacaaggagaactgttcgccgatttgtaacactcctgcatccatccaagtgggtatgcgctatgcaatgttaagctaggtcaggtcagaccaggtccaaggacagcaacttgactgtatgcaacctttaccatctttgcacagaacatacttgtagctagctagttacacttatggaccgaaaaggcaccccaccatgtctgtccggctttagagtacggccgcagaccgctgatttgccttgccaagcagtagtcacaatgcatcgcatgagcacacgggcacgggcacgggcacaggaaccattggcaaaaataccagatacactataccgacgtatatcaagcccaagtttaaaattcctaaatttccgcggggatcgactcataaaatagtaaccttctaatgcgtatctattgactaccaaccattagtgtggttgcagaaggcggaattctcccttcttcgaattcagcttgctttttcattttttattttccatttttcagtttttgtttgtgtcgaatttagccagttgcttctccaagatgaaaaaaacccctgcgcagtttctgtgctgcaagatcctaatcgacttttccaccccccacaaaagtaaatgttcttttgttacattcgcgtgggtagctagctccccgaatcttcaaaggacttagggactgcactacatcagagtgtgttcacctggtttgctgcctggtttgaaagaaaagagcagggaactcgcgggttcccggcgaataatcatgcgatagtcctttggccttccaagtcacatgtagagtagacaacagacagggagggcaggaaggatctttcactgagatcctgtatcttgttgggtaagtcggatgaaaggggaatcgtatgagattggagaggatgcggaagaggtaacgccttttgttaacttgtttaattattatggggcaggcgagagggggaggaatgtatgtgtgtgaggcgggcgagacggagccatccaggccaggtagaaatagagaaagccgaatgttagacaatatggcagcgtagtagagtaggtaggtaggcaagtactgctagcaaagaggagaagggtaagctcactcttcgcattccacaccgttagtgtgtcagtttgaacaaaaaaacaatcatcataccaattgatggactgtggactggcttttggaacggcttttcggactgcgattattcgtgaggaatcaaggtaggaatttggtcatatttacggacaacagtgggtgattcccatatggagtaggaaaacgagatcatggtatcctcagatatgttgcggaattctgttcaccgcaaagttcagggtgctctggtgggtttcggttggtctttgctttgcttctcccttgtcttgcatgttaataatagcctagcctgtgagccgaaacttagggtaggcttagtgttggaacgtacgtatgtatcacgttgacttggtttaaccaggcgacctggtagccagccatacccacacacgttttttgtatcttcagtatagttgtgaaaagtgtagcggaaatttgtggtccgagcaacagcgtctttttctagtagtgcggtcggttacttggttgacattggtatttggactttgttgctacaccattcactacttgaagtcgagtgtgaagggtatgatttctagtggtgaacacctttagttacgtaatgttttcattgctgttttacttgagatttcgattgagaaaaaggtatttaatagctcgaatcaatgtgagaacagagagaggatgttcttccctaactcgaaaggtatatgaggcttgtgtttcttaggagaattattattcttttgttatgttgcgcttgtagttggaaaaggtgaagagacaaaagctggaattgtgagcggataacaagctcaacacttgaaatttaggaaagagcagaatttggcaaaaaaaataaaaaaaaaataaacacacatactcatcgagaagctgtaccgtcgacggcgcgccatgtnngcggccgcctcgactcagtactgacaataaaaagattcttgttttcaagaacttgtcatttgtatagtttttttatattgtagttgttctattttaatcaaatgttagcgtgatttatattttttttcgcctcgacatcatctgcccagatgcgaagttaagtgcgcagaaagtaatatcatgcgtcaatcgtatgtgaatgctggtcgctatactgctgtcgattcgatactaacgccgccatccagtgtcgaaaacgagctcgggagccaactcctttcatatgctcccacctggccacccacccacacacacatacatacacaaacacaaacgatttgtttatttaaatatttattttgtacattgtcgcatagaaaatgcatatttatctgacgttcttcttcgttacgccctttcatggtttaagggatgactcaatttacactatcctgcaaggtgctacaacaatgtattagtcaggtgatcgcaaattgcatggaatatccatggtatcaccaaagaagtttcaatcttaaagtcctctggaaaacctttcttactgtgctttgaaaagaccttattcgtattcttaccctttcaataaatgaccgtggtttttttttgttatcgttataatattagaccataaaatatcgtttacgtaaacggtcgaccttgtcaacgagaaaaaaggaaacaagtccaacgttattctagaggtagccttcatagtttcaactggaactactccaaattatattttcaaaccttcaaagtatgttgaggtttactcatgtgcttaataatggggcgaaacgctctgctcttagtttaggaagaagctacttgcgtggtttcggttccatgcatggacctcgagttgctgtttcaactttaatcaaaaaagacaagaaacctaatggctttcgtggtatgttggctttatttgtaggtatcggaacactcgctgtaagcgggctttctacaaacttatacaatgatcaaaatgttaaggaagatccttggaaaagtgtgtctgttgataagtctattgacccgtttccaactgagttaaaggctcctgagttccccatttctactgaatatgttatgttaggctttggtataaggtcggttactttcattagtttcaaagtttatgggttaggtatctatgctgcaaaagaggatttgggattaatccctaaagtattggattcaaactttctttctactgcgttcattgatttcgactccagtaaaagtcatcaggagaatttgaagactgctttagacaaccctgaaacttccagaattctcattaacaacttattggatagtggaatcagattggtcgcaaaaatcacacctatcagaaacactgacttcaaccatctcaaagacggtcttgtgaaatccattcttgggcatccggatagtaaaaaggatgaagataggttaacgaatggattacaacaattacgcgatgctttctcaagaaaaggttcagtaccaaagaataacgatttattgattgaattgcaagccaacggatatttgcaagtatcctatttcgatagaaaaacaggagaatccaccacaatgggacaggtaaaagagacattgatcggtaaattactcttcagtcaatatttaagtggacctaaaccgttaagtccaagcacaaaagattctgtggtatctaaattagttacattggcttaagacacgtgtcaagcttgatatcctgcattaatgaatcggccaacgcgcggggagaggcggtttgcgtattgggcgctcttccgcttcctcgctcactgactcgctgcgctcggtcgttcggctgcggcgagcggtatcagctcactcaaaggcggtaatacggttatccacagaatcaggggataacgcaggaaagaacatgtgagcaaaaggccagcaaaaggccaggaaccgtaaaaaggccgcgttgctggcgtttttccataggctccgcccccctgacgagcatcacaaaaatcgacgctcaagtcagaggtggcgaaacccgacaggactataaagataccaggcgtttccccctggaagctccctcgtgcgctctcctgttccgaccctgccgcttaccggatacctgtccgcctttctcccttcgggaagcgtggcgctttctcatagctcacgctgtaggtatctcagttcggtgtaggtcgttcgctccaagctgggctgtgtgcacgaaccccccgttcagcccgaccgctgcgccttatccggtaactatcgtcttgagtccaacccggtaagacacgacttatcgccactggcagcagccactggtaacaggattagcagagcgaggtatgtaggcggtgctacagagttcttgaagtggtggcctaactacggctacactagaagaacagtatttggtatctgcgctctgctgaagccagttaccttcggaaaaagagttggtagctcttgatccggcaaacaaaccaccgctggtagcggtggtttttttgtttgcaagcagcagattacgcgcagaaaaaaaggatctcaagaagatcctttgatcttttctacggggtctgacgctcagtggaacgaaaactcacgttaagggattttggtcatgagattatcaaaaaggatcttcacctagatccttttaaattaaaaatgaagttttaaatcaatctaaagtatatatgagtaaacttggtctgacagttaccaatgcttaatcagtgaggcacctatctcagcgatctgtctatttcgttcatccatagttgcctgactccccgtcgtgtagataactacgatacgggagggcttaccatctggccccagtgctgcaatgataccgcgagacccacgctcaccggctccagatttatcagcaataaaccagccagccggaagggccgagcgcagaagtggtcctgcaactttatccgcctccatccagtctattaattgttgccgggaagctagagtaagtagttcgccagttaatagtttgcgcaacgttgttgccattgctacaggcatcgtggtgtcacgctcgtcgtttggtatggcttcattcagctccggttcccaacgatcaaggcgagttacatgatcccccatgttgtgcaaaaaagcggttagctccttcggtcctccgatcgttgtcagaagtaagttggccgcagtgttatcactcatggttatggcagcactgcataattctcttactgtcatgccatccgtaagatgcttttctgtgactggtgagtactcaaccaagtcattctgagaatagtgtatgcggcgaccgagttgctcttgcccggcgtcaatacgggataataccgcgccacatagcagaactttaaaagtgctcatcattggaaaacgttcttcggggcgaaaactctcaaggatcttaccgctgttgagatccagttcgatgtaacccactcgtgcacccaactgatcttcagcatcttttactttcaccagcgtttctgggtgagcaaaaacaggaaggcaaaatgccgcaaaaaagggaataagggcgacacggaaatgttgaatactcatactcttcctttttcaatattattgaagcatttatcagggttattgtctcatgagcggatacatatttgaatgtatttagaaaaataaacaaataggggttccgcgcacatttccccgaaaagtgccacctgacgtctaagaaaccattattatcatgacattaacctataaaaataggcgtatcacgaggccctttcgtctcgcgcgtttcggtgatgacggtgaaaacctctgacacatgcagctcccggagaaagaaagacgttggtctctacgctatgaactttggtaacgcttacgtcgcatctgttgctgtttattcatcatacacacagctacttacatcatttgtcgaagcttctaaatttgttggaccatcaatcattctagcgtacttgccatacaactcagaaagagacactccactagaagttttaaaagaaaccaaaattggtgtcgaaagtggttactggcctttatacaggtttaacccttacgaagaacgcgacgaccaagttttcaaattggactcctctgttatcaaacaacaactgaaggactttttagaccgagagaataagctcactcttctagctcaaaagtccccagagcttgccagaaatttgaagcattccgcctcagatgcgattcaattgaaacaagacagaagggctaaagcagcattcgatcaactcttagaaggtctctctggccctcctcttcacatttatcatgcttctgacggtggcaatgcagctaatttagcaaaaagattgggtacaagggcatctgctagaggtctaaaaactattgtactatcaatggaagacattgttctagaagagttaccaggtgaagagaatgttgtatttataacgtcaactgctggtcaaggtgaattccctcaagatggtaaggcattttgggatgctctgaagtcttctactgacctcgatttagcttctttgaatttctccgtgtttggtttaggtgactctgcatactggccacgtaaggaagacgcccattactacaacaaacccgctaaggatttgttcaagagattagaattgctttctggtcaagaactagtttctttgggattgggtgatgaccaggatgccgatggttatcaaacaggctatgctgtgtgggaagc

SEQ ID NO: 5 - DNA, 2794 bp, Artifizielle Sequenz
  Synthetische Polynukleinsäure
cgtaattctgtctttaatcattaacactgactgaaggatataattataagacaacacacagagacttttgtttgctgtttagcttacactttccagctatattgaatagcatatatatgttccagaagctacaaccaccttgaactacagcccaactcaacattgaaagttactgcctttatataccttgatacaccatttagacctccaattaaccgattgtccttgtcataatgagctagagtagcaaggtatcaacaacagtatggacatcttattgtcaactttctagtacggagggaagaatcccgaatatgttaaatctgacgcgcgggtattgctaagtcacgttgcaggcccacgcagacccgagtttctttcttacaaaagcgtgtacacacgtaaacgcgctcggtgcaccgaacggccagggtcggggttcattcggtatagagccacgcaggtaacttgccaattccaaaaaaaattaaatgacgatactagtaaccaaaggaaaggaacagatagataaaattccgagactgtcaaattaggtttttttctttttttttggcgggagtcagtgggccgaaatatgttcttggcctagaacttaatctggtttgatcatgccaatacttgcctgagtgcccgactttttgcccaccctcttgccttctgtctatccttcaaaacccacctgttttccagccgtatcttcgctcgcatctacacatactgtgccatatcttgtgtgtagccggacgtgactatgaccaaaaacaaacaaggagaactgttcgccgatttgtaacactcctgcatccatccaagtgggtatgcgctatgcaatgttaagctaggtcaggtcagaccaggtccaaggacagcaacttgactgtatgcaacctttaccatctttgcacagaacatacttgtagctagctagttacacttatggaccgaaaaggcaccccaccatgtctgtccggctttagagtacggccgcagaccgctgatttgccttgccaagcagtagtcacaatgcatcgcatgagcacacgggcacgggcacgggcacaggaaccattggcaaaaataccagatacactataccgacgtatatcaagcccaagtttaaaattcctaaatttccgcggggatcgactcataaaatagtaaccttctaatgcgtatctattgactaccaaccattagtgtggttgcagaaggcggaattctcccttcttcgaattcagcttgctttttcattttttattttccatttttcagtttttgtttgtgtcgaatttagccagttgcttctccaagatgaaaaaaacccctgcgcagtttctgtgctgcaagatcctaatcgacttttccaccccccacaaaagtaaatgttcttttgttacattcgcgtgggtagctagctccccgaatcttcaaaggacttagggactgcactacatcagagtgtgttcacctggtttgctgcctggtttgaaagaaaagagcagggaactcgcgggttcccggcgaataatcatgcgatagtcctttggccttccaagtcgcatgtagagtagacaacagacagggagggcaggaaggatctttcactgagatcctgtatcttgttgggtaagtcggatgaaaggggaatcgtatgagattggagaggatgcggaagaggtaacgccttttgttaacttgtttaattattatggggcaggcgagagggggaggaatgtatgtgtgtgaggcgggcgagacggagccatccaggccaggtagaaatagagaaagccgaatgttagacaatatggcagcgtagtagagtaggtaggtaggcaagtactgctagcaaagaggagaagggtaagctcactcttcgcattccacaccgttagtgtgtcagtttgaacaaaaaaacaatcatcataccaattgatggactgtggactggcttttggaacggcttttcggactgcgattattcgtgaggaatcaaggtaggaatttggtcatatttacggacaacagtgggtgattcccatatggagtaggaaaacgagatcatggtatcctcagatatgttgcggaattctgttcaccgcaaagttcagggtgctctggtgggtttcggttggtctttgctttgcttctcccttgtcttgcatgttaataatagcctagcctgtgagccgaaacttagggtaggcttagtgttggaacgtacatatgtatcacgttgacttggtttaaccaggcgacctggtagccagccatacccacacacgttttttgtatcttcagtatagttgtgaaaagtgtagcggaaatttgtggtccgagcaacagcgtctttttctagtagtgcggtcggttacttggttgacattggtatttggactttgttgctacaccattcactacttgaagtcgagtgtgaagggtatgatttctagtggtgaacacctttagttacgtaatgttttcattgctgttttacttgagatttcgattgagaaaaaggtatttaatagctcgaatcaatgtgagaacagagagaggatgttcttccctaactcgaaaggtatatgaggcttgtgtttcttaggagaattattattcttttgttatgttgcgcttgtagttggaaaaggtgaagagacaaaagctggaattgtgagcggataacaagctcaacacttgaaatttaggaaagagcagaatttggcaaaaaaaataaaaaaaaaataaacacacatactcatcgagaagctgt

SEQ ID NO: 6 - DNA, 2329 bp, Artifizielle Sequenz
  Synthetische Polynukleinsäure
cgtaattctgtctttaatcattaacactgactgaaggatataattataagacaacacacagagacttttgtttgctgtttagcttacactttccagctatattgaatagcatatatatgttccagaagctacaaccaccttgaactacagcccaactcaacattgaaagttactgcctttatataccttgatacaccatttagacctccaattaaccgattgtccttgtcataatgagctagagtagcaaggtatcaacaacagtatggacatcttattgtcaactttctagtacggagggaagaatcccgaatatgttaaatctgacgcgcgggtattgctaagtcacgttgcaggcccacgcagacccgagtttctttcttacaaaagcgtgtacacacgtaaacgcgctcggtgcaccgaacggccagggtcggggttcattcggtatagagccacgcaggtaacttgccaattccaaaaaaaattaaatgacgatactagtaaccaaaggaaaggaacagatagataaaattccgagactgtcaaattaggtttttttctttttttttggcgggagtcagtgggccgaaatatgttcttggcctagaacttaatctggtttgatcatgccaatacttgcctgagtgcccgactttttgcccaccctcttgccttctgtctatccttcaaaacccacctgttttccagccgtatcttcgctcgcatctacacatactgtgccatatcttgtgtgtagccggacgtgactatgaccaaaaacaaacaaggagaactgttcgccgatttgtaacactcctgcatccatccaagtgggtatgcgctatgcaatgttaagctaggtcaggtcagaccaggtccaaggacagcaacttgactgtatgcaacctttaccatctttgcacagaacatacttgtagctagctagttacacttatggaccgaaaaggcaccccaccatgtctgtccggctttagagtacggccgcagaccgctgatttgccttgccaagcagtagtcacaatgcatcgcatgagcacacgggcacgggcacgggcacaggaaccattggcaaaaataccagatacactataccgacgtatatcaagcccaagtttaaaattcctaaatttccgcggggatcgactcataaaatagtaaccttctaatgcgtatctattgactaccaaccattagtgtggttgcagaaggcggaattcgtcgacgaacttgtttaattattatggggcaggcgagagggggaggaatgtatgtgtgtgaggcgggcgagacggagccatccaggccaggtagaaatagagaaagccgaatgttagacaatatggcagcgtagtagagtaggtaggtaggcaagtactgctagcaaagaggagaagggtaagctcactcttcgcattccacaccgttagtgtgtcagtttgaacaaaaaaacaatcatcataccaattgatggactgtggactggcttttggaacggcttttcggactgcgattattcgtgaggaatcaaggtaggaatttggtcatatttacggacaacagtgggtgattcccatatggagtaggaaaacgagatcatggtatcctcagatatgttgcggaattctgttcaccgcaaagttcagggtgctctggtgggtttcggttggtctttgctttgcttctcccttgtcttgcatgttaataatagcctagcctgtgagccgaaacttagggtaggcttagtgttggaacgtacatatgtatcacgttgacttggtttaaccaggcgacctggtagccagccatacccacacacgttttttgtatcttcagtatagttgtgaaaagtgtagcggaaatttgtggtccgagcaacagcgtctttttctagtagtgcggtcggttacttggttgacattggtatttggactttgttgctacaccattcactacttgaagtcgagtgtgaagggtatgatttctagtggtgaacacctttagttacgtaatgttttcattgctgttttacttgagatttcgattgagaaaaaggtatttaatagctcgaatcaatgtgagaacagagagaggatgttcttccctaactcgaaaggtatatgaggcttgtgtttcttaggagaattattattcttttgttatgttgcgcttgtagttggaaaaggtgaagagacaaaagctggaattgtgagcggataacaagctcaacacttgaaatttaggaaagagcagaatttggcaaaaaaaataaaaaaaaaataaacacacatactcatcgagaagctgt

SEQ ID NO: 7 - DNA, 1638 bp, Artifizielle Sequenz
  Synthetische Polynukleinsäure
gcggggatcgactcataaaatagtaaccttctaatgcgtatctattgactaccaaccattagtgtggttgcagaaggcggaattctcccttcttcgaattcagcttgctttttcattttttattttccatttttcagtttttgtttgtgtcgaatttagccagttgcttctccaagatgaaaaaaacccctgcgcagtttctgtgctgcaagatcctaatcgacttttccaccccccacaaaagtaaatgttcttttgttacattcgcgtgggtagctagctccccgaatcttcaaaggacttagggactgcactacatcagagtgtgttcacctggtttgctgcctggtttgaaagaaaagagcagggaactcgcgggttcccggcgaataatcatgcgatagtcctttggccttccaagtcgcatgtagagtagacaacagacagggagggcaggaaggatctttcactgagatcctgtatcttgttgggtaagtcggatgaaaggggaatcgtatgagattggagaggatgcggaagaggtaacgccttttgttaacttgtttaattattatggggcaggcgagagggggaggaatgtatgtgtgtgaggcgggcgagacggagccatccaggccaggtagaaatagagaaagccgaatgttagacaatatggcagcgtagtagagtaggtaggtaggcaagtactgctagcaaagaggagaagggtaagctcactcttcgcattccacaccgttagtgtgtcagtttgaacaaaaaaacaatcatcataccaattgatggactgtggactggcttttggaacggcttttcggactgcgattattcgtgaggaatcaaggtaggaatttggtcatatttacggacaacagtgggtgattcccatatggagtaggaaaacgagatcatggtatcctcagatatgttgcggaattctgttcaccgcaaagttcagggtgctctggtgggtttcggttggtctttgctttgcttctcccttgtcttgcatgttaataatagcctagcctgtgagccgaaacttagggtaggcttagtgttggaacgtacatatgtatcacgttgacttggtttaaccaggcgacctggtagccagccatacccacacacgttttttgtatcttcagtatagttgtgaaaagtgtagcggaaatttgtggtccgagcaacagcgtctttttctagtagtgcggtcggttacttggttgacattggtatttggactttgttgctacaccattcactacttgaagtcgagtgtgaagggtatgatttctagtggtgaacacctttagttacgtaatgttttcattgctgttttacttgagatttcgattgagaaaaaggtatttaatagctcgaatcaatgtgagaacagagagaggatgttcttccctaactcgaaaggtatatgaggcttgtgtttcttaggagaattattattcttttgttatgttgcgcttgtagttggaaaaggtgaagagacaaaagctggaattgtgagcggataacaagctcaacacttgaaatttaggaaagagcagaatttggcaaaaaaaataaaaaaaaaataaacacacatactcatcgagaagctgt

SEQ ID NO: 8 - DNA, 1081 bp, Artifizielle Sequenz
  Synthetische Polynukleinsäure
aacttgtttaattattatggggcaggcgagagggggaggaatgtatgtgtgtgaggcgggcgagacggagccatccaggccaggtagaaatagagaaagccgaatgttagacaatatggcagcgtagtagagtaggtaggtaggcaagtactgctagcaaagaggagaagggtaagctcactcttcgcattccacaccgttagtgtgtcagtttgaacaaaaaaacaatcatcataccaattgatggactgtggactggcttttggaacggcttttcggactgcgattattcgtgaggaatcaaggtaggaatttggtcatatttacggacaacagtgggtgattcccatatggagtaggaaaacgagatcatggtatcctcagatatgttgcggaattctgttcaccgcaaagttcagggtgctctggtgggtttcggttggtctttgctttgcttctcccttgtcttgcatgttaataatagcctagcctgtgagccgaaacttagggtaggcttagtgttggaacgtacatatgtatcacgttgacttggtttaaccaggcgacctggtagccagccatacccacacacgttttttgtatcttcagtatagttgtgaaaagtgtagcggaaatttgtggtccgagcaacagcgtctttttctagtagtgcggtcggttacttggttgacattggtatttggactttgttgctacaccattcactacttgaagtcgagtgtgaagggtatgatttctagtggtgaacacctttagttacgtaatgttttcattgctgttttacttgagatttcgattgagaaaaaggtatttaatagctcgaatcaatgtgagaacagagagaggatgttcttccctaactcgaaaggtatatgaggcttgtgtttcttaggagaattattattcttttgttatgttgcgcttgtagttggaaaaggtgaagagacaaaagctggaattgtgagcggataacaagctcaacacttgaaatttaggaaagagcagaatttggcaaaaaaaataaaaaaaaaataaacacacatactcatcgagaagctgt

SEQ ID NO: 9 - DNA, 20 bp, Artifizielle Sequenz
  Primer
gagcccaccacctgctcctg

SEQ ID NO: 10 - DNA, 25 bp, Artificial sequrence
  Primer
ctgatgtattgcgctccttactaac

SEQ ID NO: 11 - DNA, 20 bp, Artifizielle Sequenz
  Primer
cccagatgcgaagttaagtg

SEQ ID NO: 12 - DNA, 29 bp, Artifizielle Sequenz
  Primer
tacaacagatcacgtgatctttttgtaag

SEQ ID NO: 13 - DNA, 28 bp, Artifizielle Sequenz
  Primer
gatttcgtaaccctattgttcatgaatg

SEQ ID NO: 14 - DNA, 475 bp, Artifizielle Sequenz
  Synthetische Polynukleinsäure
ttctcccttcttcgaattcagcttgctttttcattttttattttccatttttcagtttttgtttgtgtcgaatttagccagttgcttctccaagatgaaaaaaacccctgcgcagtttctgtgctgcaagatcctaatcgacttttccaccccccacaaaagtaaatgttcttttgttacattcgcgtgggtagctagctccccgaatcttcaaaggacttagggactgcactacatcagagtgtgttcacctggtttgctgcctggtttgaaagaaaagagcagggaactcgcgggttcccggcgaataatcatgcgatagtcctttggccttccaagtcgcatgtagagtagacaacagacagggagggcaggaaggatctttcactgagatcctgtatcttgttgggtaagtcggatgaaaggggaatcgtatgagattggagaggatgcggaagaggtaacgccttttgtt

SEQ ID NO: 15 - DNA, 52 bp, Artifizielle Sequenz
  Primer
tatagggcgaattggagctccgccggcggaagaggtaacgccttttgttaac

SEQ ID NO: 16 - DNA, 44 bp, Artifizielle Sequenz
  Primer
ctaaacggaactcgcatttaaatctcgttttcgacactggatgg

SEQ ID NO: 17 - DNA, 55 bp, Artifizielle Sequenz
  Primer
gcgagttccgtttagacgcgtttaaacttgtttaattattatggggcaggcgaga

SEQ ID NO: 18 - DNA, 40 bp, Artifizielle Sequenz
  Primer
cggggaatgcgctgcttttcgacactggatggcggcgtta

SEQ ID NO: 19 - DNA, 43 bp, Artifizielle Sequenz
  Primer
gcagcgcattccccgggtaccgctctcgactaggtgattagcg

SEQ ID NO: 20 - DNA, 51 bp, Artifizielle Sequenz
  Primer
aaaagctgggtaccgggcccactagtcgagagttaaccgtgactacagcta

SEQ ID NO: 21 - DNA, 11582 bp, Artifizielle Sequenz
  Synthetische Polynukleinsäure
ggacgcgccctgtagcggcgcattaagcgcggcgggtgtggtggttacgcgcagcgtgaccgctacacttgccagcgccctagcgcccgctcctttcgctttcttcccttcctttctcgccacgttcgccggctttccccgtcaagctctaaatcgggggctccctttagggttccgatttagtgctttacggcacctcgaccccaaaaaacttgattagggtgatggttcacgtagtgggccatcgccctgatagacggtttttcgccctttgacgttggagtccacgttctttaatagtggactcttgttccaaactggaacaacactcaaccctatctcggtctattcttttgatttataagggattttgccgatttcggcctattggttaaaaaatgagctgatttaacaaaaatttaacgcgaattttaacaaaatattaacgtttacaatttcgcgccattcgccattcaggctgcgcaactgttgggaagggcgatcggtgcgggcctcttcgctattacgccagctggcgaaagggggatgtgctgcaaggcgattaagttgggtaacgccagggttttcccagtcacgacgttgtaaaacgacggccagtgaattgtaatacgactcactatagggcgaattggagctccgccggcggaagaggtaacgccttttgttaacttgtttaattattatggggcaggcgagagggggaggaatgtatgtgtgtgaggcgggcgagacggagccatccaggccaggtagaaatagagaaagccgaatgttagacaatatggcagcgtagtagagtaggtaggtaggcaagtactgctagcaaagaggagaagggtaagctcactcttcgcattccacaccgttagtgtgtcagtttgaacaaaaaaacaatcatcataccaattgatggactgtggactggcttttggaacggcttttcggactgcgattattcgtgaggaatcaaggtaggaatttggtcatatttacggacaacagtgggtgattcccatatggagtaggaaaacgagatcatggtatcctcagatatgttgcggaattctgttcaccgcaaagttcagggtgctctggtgggtttcggttggtctttgctttgcttctcccttgtcttgcatgttaataatagcctagcctgtgagccgaaacttagggtaggcttagtgttggaacgtacatatgtatcacgttgacttggtttaaccaggcgacctggtagccagccatacccacacacgttttttgtatcttcagtatagttgtgaaaagtgtagcggaaatttgtggtccgagcaacagcgtctttttctagtagtgcggtcggttacttggttgacattggtatttggactttgttgctacaccattcactacttgaagtcgagtgtgaagggtatgatttctagtggtgaacacctttagttacgtaatgttttcattgctgttttacttgagatttcgattgagaaaaaggtatttaatagctcgaatcaatgtgagaacagagagaagatgttcttccctaactcgaaaggtatatgaggcttgtgtttcttaggagaattattattcttttgttatgttgcgcttgtagttggaaaaggtgaagagacaaaagctggaattgtgagcggataacaagctcaacacttgaaatttaggaaagagcagaatttggcaaaaaaaataaaaaaaaaataaacacacatactcatcgagaagctgtaccgtcgacggcgcgccgatgtccaacttacaagaccaaacccaacaaatcgtcccttttatcagatccttattaatgcctactaccggtcctgcttctattcctgatgacaccttggaaaaacacaccttgagatccgaaacttcaacctataacttgactgtcggtgacactggttctggtttaatcgttttcttccctggttttcctggttcaattgtcggtgcccactataccttacaaggtaacggtaactataagttcgatcaaatgttgttgaccgcccaaaatttgcctgcctcctataactattgtagattggtttctagatctttaaccgtcagatcatccactttgcctggtggtgtctatgctttgaacggtacaatcaacgctgtcacatttcaaggttccttgtccgaattgaccgatgtctcctataacggtttaatgtccgctactgccaatatcaatgacaaaattggtaacgtcttagtcggtgaaggtgttactgttttgagtttgccaacctcttatgacttgggttatgtcagattgggtgaccctattcctgctatcggtttagacccaaaaatggttgccacttgtgactctagtgatagaccaagagtctataccatcactgctgccgatgactatcaattctcctcccaatatcaacctggtggtgtcactatcaccttgttctctgccaacatcgacgctataacatctttgtccgtcggtggtgaattggtattccaaacctccgtccatggtttagtattgggtgccaccatctatttgattggtttcgacggtacaaccgtcattactagagccgttgctgccaacaatggtttaaccactggtactgacaacttgatgccattcaacttggtaatccctaccaacgaaatcacacaaccaatcacatccatcaaattggaaattgtcacctccaaatccggtggtcaagccggtgaccaaatgtcatggagtgctagaggttcattagccgtaaccatccacggtggtaactatcctggtgccttgagacctgtcactttagtcgcctatgaaagagttgctactggttccgtcgttactgttgccggtgtttcaaacttcgaattgatcccaaacccagaattggccaaaaacttggttaccgaatatggtagattcgaccctggtgctatgaactatacaaaattgatcttatccgaaagagacagattgggtatcaaaactgtctggcctactagagaatataccgactttagagaatatttcatggaagtcgccgacttaaattccccattgaaaatcgccggtgcctttggttttaaggacatcattagagccattagaagaatagccgtctgagcggccgcctcgactcagtactgacaataaaaagattcttgttttcaagaacttgtcatttgtatagtttttttatattgtagttgttctattttaatcaaatgttagcgtgatttatattttttttcgcctcgacatcatctgcccagatgcgaagttaagtgcgcagaaagtaatatcatgcgtcaatcgtatgtgaatgctggtcgctatactgctgtcgattcgatactaacgccgccatccagtgtcgaaaacgagatttaaatgcgagttccgtttagacgcgtttaaacttgtttaattattatggggcaggcgagagggggaggaatgtatgtgtgtgaggcgggcgagacggagccatccaggccaggtagaaatagagaaagccgaatgttagacaatatggcagcgtagtagagtaggtaggtaggcaagtactgctagcaaagaggagaagggtaagctcactcttcgcattccacaccgttagtgtgtcagtttgaacaaaaaaacaatcatcataccaattgatggactgtggactggcttttggaacggcttttcggactgcgattattcgtgaggaatcaaggtaggaatttggtcatatttacggacaacagtgggtgattcccatatggagtaggaaaacgagatcatggtatcctcagatatgttgcggaattctgttcaccgcaaagttcagggtgctctggtgggtttcggttggtctttgctttgcttctcccttgtcttgcatgttaataatagcctagcctgtgagccgaaacttagggtaggcttagtgttggaacgtacatatgtatcacgttgacttggtttaaccaggcgacctggtagccagccatacccacacacgttttttgtatcttcagtatagttgtgaaaagtgtagcggaaatttgtggtccgagcaacagcgtctttttctagtagtgcggtcggttacttggttgacattggtatttggactttgttgctacaccattcactacttgaagtcgagtgtgaagggtatgatttctagtggtgaacacctttagttacgtaatgttttcattgctgttttacttgagatttcgattgagaaaaaggtatttaatagctcgaatcaatgtgagaacagagagaagatgttcttccctaactcgaaaggtatatgaggcttgtgtttcttaggagaattattattcttttgttatgttgcgcttgtagttggaaaaggtgaagagacaaaagctggaattgtgagcggataacaagctcaacacttgaaatttaggaaagagcagaatttggcaaaaaaaataaaaaaaaaataaacacacatactcatcgagaagctgtaccgtcgacggcgcgccgatgtccaacttacaagaccaaacccaacaaatcgtcccttttatcagatccttattaatgcctactaccggtcctgcttctattcctgatgacaccttggaaaaacacaccttgagatccgaaacttcaacctataacttgactgtcggtgacactggttctggtttaatcgttttcttccctggttttcctggttcaattgtcggtgcccactataccttacaaggtaacggtaactataagttcgatcaaatgttgttgaccgcccaaaatttgcctgcctcctataactattgtagattggtttctagatctttaaccgtcagatcatccactttgcctggtggtgtctatgctttgaacggtacaatcaacgctgtcacatttcaaggttccttgtccgaattgaccgatgtctcctataacggtttaatgtccgctactgccaatatcaatgacaaaattggtaacgtcttagtcggtgaaggtgttactgttttgagtttgccaacctcttatgacttgggttatgtcagattgggtgaccctattcctgctatcggtttagacccaaaaatggttgccacttgtgactctagtgatagaccaagagtctataccatcactgctgccgatgactatcaattctcctcccaatatcaacctggtggtgtcactatcaccttgttctctgccaacatcgacgctataacatctttgtccgtcggtggtgaattggtattccaaacctccgtccatggtttagtattgggtgccaccatctatttgattggtttcgacggtacaaccgtcattactagagccgttgctgccaacaatggtttaaccactggtactgacaacttgatgccattcaacttggtaatccctaccaacgaaatcacacaaccaatcacatccatcaaattggaaattgtcacctccaaatccggtggtcaagccggtgaccaaatgtcatggagtgctagaggttcattagccgtaaccatccacggtggtaactatcctggtgccttgagacctgtcactttagtcgcctatgaaagagttgctactggttccgtcgttactgttgccggtgtttcaaacttcgaattgatcccaaacccagaattggccaaaaacttggttaccgaatatggtagattcgaccctggtgctatgaactatacaaaattgatcttatccgaaagagacagattgggtatcaaaactgtctggcctactagagaatataccgactttagagaatatttcatggaagtcgccgacttaaattccccattgaaaatcgccggtgcctttggttttaaggacatcattagagccattagaagaatagccgtctgagcggccgcctcgactcagtactgacaataaaaagattcttgttttcaagaacttgtcatttgtatagtttttttatattgtagttgttctattttaatcaaatgttagcgtgatttatattttttttcgcctcgacatcatctgcccagatgcgaagttaagtgcgcagaaagtaatatcatgcgtcaatcgtatgtgaatgctggtcgctatactgctgtcgattcgatactaacgccgccatccagtgtcgaaaagcagcgcattccccgggtaccgctctcgactaggtgattagcggggggagatgaaaagtgttacaacgtttgtctcgcaccctgtaaccttatactattgaacaaaccaactaaaacaaaaaaaaaaactactatcaacaaaacttcgagctttaacccaagttatcaattgtttaaaatgactctaaatttctaatacccttattctttctattcttcttcttctttttaactatatctacttatattctattaaatatcacatttacgtttgtattacatgactactcttgtcaaccaggacgttagtggtccataacctcaggttcagccggctcatagtcttccgaatcgtacattattcatcgctcggacctctccattccgttattttatccactctttgttcctctcaattcaagaattattcactttaaccacttcaacgaaatcaaataaaactccgtcgaatcagtacagtcaggaatcaccaccctggacactcccttccattgtgtttgtgtttgtgtttgtactttcattcattgtccctttttgacaatataaaggttaaacagagagctatagtatatcttgggacaattgtgatttagtcactttgaaagtgttattatttgatccagtgtacacaatatctcggcaggacggcaccatggcttgccttattcctgagaatttaaggaaccccaaaaaggttcacgaaaatagattgcctactagggcttactactatgatcaggatattttcgaatctctcaatgggccttgggcttttgcgttgtttgatgcacctcttgacgctccggatgctaagaatttagactgggaaacggcaaagaaatggagcaccatttctgtgccatcccattgggaacttcaggaagactggaagtacggtaaaccaatttacacgaacgtacagtaccctatcccaatcgacatcccaaatcctcccactgtaaatcctactggtgtttatgctagaacttttgaattagattcgaaatcgattgagtcgttcgagcacagattgagatttgagggtgtggacaattgttacgagctttatgttaatggtcaatatgtgggtttcaataaggggtcccgtaacggggctgaatttgatatccaaaagtacgtttctgagggcgaaaacttagtggtcgtcaaggttttcaagtggtccgattccacttatatcgaggaccaagatcaatggtggctctctggtatttacagagacgtttctttactaaaattgcctaagaaggcccatattgaagacgttagggtcactacaacttttgtggactctcagtatcaggatgcagagctttctgtgaaagttgatgtccagggttcttcttatgatcacatcaatttcacactttacgaacctgaagatggatctaaagtttacgatgcaagctctttgttgaacgaggagaatgggaacacgactttttcaactaaagaatttatttccttctccaccaaaaagaacgaagaaacagctttcaagatcaacgtcaaggccccagaacattggaccgcagaaaatcctactttgtacaagtaccagttggatttaattggatctgatggcagtgtgattcaatctattaagcaccatgttggtttcagacaagtggagttgaaggacggtaacattactgttaatggcaaagacattctctttagaggtgtcaacagacatgatcaccatccaaggttcggtagagctgtgccattagattttgttgttagggacttgattctaatgaagaagtttaacatcaatgctgttcgtaactcgcattatccaaaccatcctaaggtgtatgacctcttcgataagctgggcttctgggtcattgacgaggcagatcttgaaactcatggtgttcaagagccatttaatcgtcatacgaacttggaggctgaatatccagatactaaaaataaactctacgatgttaatgcccattacttatcagataatccagagtacgaggtcgcgtacttagacagagcttcccaacttgtcctaagagatgtcaatcatccttcgattattatctggtccttgggtaacgaagcttgttatggcagaaaccacaaagccatgtacaagttaattaaacaattggatcctaccagacttgtgcattatgagggtgacttgaacgctttgagtgcagatatctttagtttcatgtacccaacatttgaaattatggaaaggtggaggaagaaccacactgatgaaaatggtaagtttgaaaagcctttgatcttgtgtgagtacggccatgcaatgggtaacggtcctggctctttgaaagaatatcaagagttgttctacaaggagaagttttaccaaggtggctttatctgggaatgggcaaatcacggtattgaattcgaagatgttagtactgcagatggtaagttgcataaagcttatgcttatggtggtgactttaaggaagaggttcatgacggagtgttcatcatggatggtttgtgtaacagtgagcataatcctactccgggccttgtagagtataagaaggttattgaacccgttcatattaaaattgcgcacggatctgtaacaatcacaaataagcacgacttcattacgacagaccacttattgtttatcgacaaggacacgggaaagacaatcgacgttccatctttaaagccagaagaatctgttactattccttctgatacaacttatgttgttgccgtgttgaaagatgatgctggtgttctaaaggcaggtcatgaaattgcctggggccaagctgaacttccattgaaggtacccgattttgttacagagacagcagaaaaagctgcgaagatcaacgacggtaaacgttatgtctcagttgaatccagtggattgcattttatcttggacaaattgttgggtaaaattgaaagcctaaaggtcaagggtaaggaaatttccagcaagtttgagggttcttcaatcactttctggagacctccaacgaataatgatgaacctagggactttaagaactggaagaagtacaatattgatttaatgaagcaaaacatccatggagtgagtgtcgaaaaaggttctaatggttctctagctgtagtcacggttaactctcgactagtgggcccggtacccagcttttgttccctttagtgagggttaattccgagcttggcgtaatcatggtcatagctgtttcctgtgtgaaattgttatccgctcacaattccacacaacatacgagccggaagcataaagtgtaaagcctggggtgcctaatgagtgagctaactcacattaattgcgttgcgctcactgcccgctttccagtcgggaaacctgtcgtgccagctgcattaatgaatcggccaacgcgcggggagaggcggtttgcgtattgggcgctcttccgcttcctcgctcactgactcgctgcgctcggtcgttcggctgcggcgagcggtatcagctcactcaaaggcggtaatacggttatccacagaatcaggggataacgcaggaaagaacatgtgagcaaaaggccagcaaaaggccaggaaccgtaaaaaggccgcgttgctggcgtttttccataggctccgcccccctgacgagcatcacaaaaatcgacgctcaagtcagaggtggcgaaacccgacaggactataaagataccaggcgtttccccctggaagctccctcgtgcgctctcctgttccgaccctgccgcttaccggatacctgtccgcctttctcccttcgggaagcgtggcgctttctcatagctcacgctgtaggtatctcagttcggtgtaggtcgttcgctccaagctgggctgtgtgcacgaaccccccgttcagcccgaccgctgcgccttatccggtaactatcgtcttgagtccaacccggtaagacacgacttatcgccactggcagcagccactggtaacaggattagcagagcgaggtatgtaggcggtgctacagagttcttgaagtggtggcctaactacggctacactagaaggacagtatttggtatctgcgctctgctgaagccagttaccttcggaaaaagagttggtagctcttgatccggcaaacaaaccaccgctggtagcggtggtttttttgtttgcaagcagcagattacgcgcagaaaaaaaggatctcaagaagatcctttgatcttttctacggggtctgacgctcagtggaacgaaaactcacgttaagggattttggtcatgagattatcaaaaaggatcttcacctagatccttttaaattaaaaatgaagttttaaatcaatctaaagtatatatgagtaaacttggtctgacagttaccaatgcttaatcagtgaggcacctatctcagcgatctgtctatttcgttcatccatagttgcctgactccccgtcgtgtagataactacgatacgggagggcttaccatctggccccagtgctgcaatgataccgcgagacccacgctcaccggctccagatttatcagcaataaaccagccagccggaagggccgagcgcagaagtggtcctgcaactttatccgcctccatccagtctattaattgttgccgggaagctagagtaagtagttcgccagttaatagtttgcgcaacgttgttgccattgctacaggcatcgtggtgtcacgctcgtcgtttggtatggcttcattcagctccggttcccaacgatcaaggcgagttacatgatcccccatgttgtgcaaaaaagcggttagctccttcggtcctccgatcgttgtcagaagtaagttggccgcagtgttatcactcatggttatggcagcactgcataattctcttactgtcatgccatccgtaagatgcttttctgtgactggtgagtactcaaccaagtcattctgagaatagtgtatgcggcgaccgagttgctcttgcccggcgtcaatacgggataataccgcgccacatagcagaactttaaaagtgctcatcattggaaaacgttcttcggggcgaaaactctcaaggatcttaccgctgttgagatccagttcgatgtaacccactcgtgcacccaactgatcttcagcatcttttactttcaccagcgtttctgggtgagcaaaaacaggaaggcaaaatgccgcaaaaaagggaataagggcgacacggaaatgttgaatactcatactcttcctttttcaatattattgaagcatttatcagggttattgtctcatgagcggatacatatttgaatgtatttagaaaaataaacaaataggggttccgcgcacatttccccgaaaagtgccacctg

SEQ ID NO: 22 - DNA, 29 bp, Artifizielle Sequenz
  Primer
gacatcactgtctcttccccttaatgatc

SEQ ID NO: 23 - DNA, 29 bp, Artifizielle Sequenz
  Primer
tcagcaagcatcaataatccccttggttc

SEQ ID NO: 24 - DNA, 28 bp, Artifizielle Sequenz
  Primer
gaaagaaagacgttggtctctacgcttg

SEQ ID NO: 25 - DNA, 29 bp, Artifizielle Sequenz
  Primer
agattataagttcctggggctttacccac